European Patent Application EP 4 696 708 A1, published February 18, 2026. Title: PEPTIDE TYROSINE- TYROSINE ANALOG AND USE THEREOF. Applicant: THE UNITED BIO-TECHNOLOGY (HENGQIN) CO., LTD. The sequence listing filed with the application follows.

SEQUENCE LISTING (7 sequences)

SEQ ID NO: 1 - protein, 36 aa, Homo sapiens
YPIKPEAPGEDASPEELNRYYASLRHYLNLVTRQRY

SEQ ID NO: 2 - protein, 34 aa, Homo sapiens
IKPEAPGEDASPEELNRYYASLRHYLNLVTRQRY

SEQ ID NO: 3 - protein, 34 aa, synthetic construct
  MOD_RES 10: note = Aib
  MOD_RES 20: note = Aib
PKPEKPEEDXSPEEWQRYYXSLRHYLNWLTRQRY

SEQ ID NO: 4 - protein, 34 aa, synthetic construct
  MOD_RES 8: note = Aib
PKPEKPEXDASPEEWQRYYAELRHYLNWLTRQRY

SEQ ID NO: 5 - protein, 34 aa, synthetic construct
  MOD_RES 8: note = Aib
  MOD_RES 20: note = Aib
PKPEKPEXDASPEEWQRYYXELRHYLNWLTRQRY

SEQ ID NO: 6 - protein, 34 aa, synthetic construct
PKPEKPGKDASPEEWNRYYADLRHYLNWLTRQRY

SEQ ID NO: 7 - protein, 31 aa, synthetic construct
HAEGTFTSDVSSYLEGQAAKEFIAWLVRGRG